European Patent Specification EP 4 496 802 B1, published September 24, 2025. Title: Peptides and compositions for use in cosmetics, food and medicine. Applicant: LIPOTRUE, S.L. Application IB. The sequence listing filed with the application follows.

SEQUENCE LISTING (3 sequences)

SEQ ID NO: 1 - skipped

SEQ ID NO: 2 - protein, 7 aa, synthetic construct
  REGION 1..7: note = Artificially synthesized sequence; note (original language) = Secuencia sintetizada artificialmente
  source 1..7: organism (original language) = Construccion sintetica
GYYELND

SEQ ID NO: 3 - protein, 7 aa, synthetic construct
  REGION 1..7: note = Artificially synthesized sequence; note (original language) = Secuencia sintetizada artificialmente
  source 1..7: organism (original language) = Construccion sintetica
GNELLDY